European Patent Specification EP 3 461 889 B1, published January 29, 2025. Title: Compositions for Increasing Polypeptide Stability and Activity, and Related Methods. Applicant: Solis BioDyne OÜ. Application EP. The sequence listing filed with the application follows.

SEQUENCE LISTING (31 sequences)

SEQ ID NO: 1 - protein, 42 aa, Artificial Sequence
  source: /note="Description of Artificial Sequence: Synthetic polypeptide"
MIDLQRPSAATMVDDLQRPHHHHHHPWDYKDDDDKPRWNSGW

SEQ ID NO: 2 - protein, 870 aa, Artificial Sequence
  source: /note="Description of Artificial Sequence: Synthetic polypeptide"
MIDLQRPSAATMVDDLQRPHHHHHHPWDYKDDDDKPRWNSGWLPLFEPKGRVLLVDGHHLAYRTFHALKGLTTSRGEPVQAVYGFAKSLLKALKEDGDAVIVVFDAKAPSFRHEAYGGYKAGRAPTPEDFPRQLALIKELVDLLGLARLEVPGYEADDVLASLAKKAEKEGYEVRILTADKDLYQLLSDRIHVLHPEGYLITPAWLWEKYGLRPDQWADYRALTGDESDNLPGVKGIGEKTARKLLEEWGSLEALLKNLDRLKPAIREKILAHMDDLKLSWDLAKVRTDLPLEVDFAKRREPDRERLRAFLERLEFGSLLHEFGLLESPKALEEAPWPPPEGAFVGFVLSRKEPMWADLLALAAARGGRVHRAPEPYKALRDLKEARGLLAKDLSVLALREGLGLPPGDDPMLLAYLLDPSNTTPEGVARRYGGEWTEEAGERAALSERLFANLWGRLEGEERLLWLYREVERPLSAVLAHMEATGVRLDVAYLRALSLEVAEEIARLEAEVFRLAGHPFNLNSRDQLERVLFDELGLPAIGKTEKTGKRSTSAAVLEALREAHPIVEKILQYRELTKLKSTYIDPLPDLIHPRTGRLHTRFNQTATATGRLSSSDPNLQNIPVRTPLGQRIRRAFIAEEGWLLVALDYSQIELRVLAHLSGDENLIRVFQEGRDIHTETASWMFGVPREAVDPLMRRAAKTINFGVLYGMSAHRLSQELAIPYEEAQAFIERYFQSFPKVRAWIEKTLEEGRRRGYVETLFGRRRYVPDLEARVKSVREAAERMAFNMPVQGTAADLMKLAMVKLFPRLEEMGARMLLQVHDELVLEAPKERAEAVARLAKEVMEGVYPLAVPLEVEVGIGEDWLSAKE

SEQ ID NO: 3 - DNA, 141 bp, Artificial Sequence
  source: /note="Description of Artificial Sequence: Synthetic polynucleotide"
acacaggaaacagcgatgatcgacctgcagcggccatccgccgccaccatggtcgacgacctgcagcggccgcaccatcaccatcaccatccatgggattacaaggacgacgatgacaagccgcggtggaattcggggtgg

SEQ ID NO: 4 - DNA, 2637 bp, Artificial Sequence
  source: /note="Description of Artificial Sequence: Synthetic polynucleotide"
acacaggaaacagcgatgatcgacctgcagcggccatccgccgccaccatggtcgacgacctgcagcggccgcaccatcaccatcaccatccatgggattacaaggacgacgatgacaagccgcggtggaattcggggtggctgcccctctttgagcccaagggccgggtcctcctggtggacggccaccacctggcctaccgcaccttccacgccctgaagggcctcaccaccagccggggggagccggtgcaggcggtctacggcttcgccaagagcctcctcaaggccctcaaggaggacggggacgcggtgatcgtggtctttgacgccaaggccccctccttccgccacgaggcctacggggggtacaaggcgggccgggcccccacgccggaggactttccccggcaactcgccctcatcaaggagctggtggacctcctggggctggcgcgcctcgaggtcccgggctacgaggcggacgacgtcctggccagcctggccaagaaggcggaaaaggagggctacgaggtccgcatcctcaccgccgacaaagacctttaccagctcctttccgaccgcatccacgtcctccaccccgaggggtacctcatcaccccggcctggctttgggaaaagtacggcctgaggcccgaccagtgggccgactaccgggccctgaccggggacgagtccgacaaccttcccggggtcaagggcatcggggagaagacggcgaggaagcttctggaggagtgggggagcctggaagccctcctcaagaacctggaccggctgaagcccgccatccgggagaagatcctggcccacatggacgatctgaagctctcctgggacctggccaaggtgcgcaccgacctgcccctggaggtggacttcgccaaaaggcgggagcccgaccgggagaggcttagggcctttctggagaggcttgagtttggcagcctcctccacgagttcggccttctggaaagccccaaggccctggaggaggccccctggcccccgccggaaggggccttcgtgggctttgtgctttcccgcaaggagcccatgtgggccgatcttctggccctggccgccgccagggggggccgggtccaccgggcccccgagccttataaagccctcagggacctgaaggaggcgcgggggcttctcgccaaagacctgagcgttctggccctgagggaaggccttggcctcccgcccggcgacgaccccatgctcctcgcctacctcctggacccttccaacaccacccccgagggggtggcccggcgctacggcggggagtggacggaggaggcgggggagcgggccgccctttccgagaggctcttcgccaacctgtgggggaggcttgagggggaggagaggctcctttggctttaccgggaggtggagaggcccctttccgctgtcctggcccacatggaggccacgggggtgcgcctggacgtggcctatctcagggccttgtccctggaggtggccgaggagatcgcccgcctcgaggccgaggtcttccgcctggccggccaccccttcaacctcaactcccgggaccagctggaaagggtcctctttgacgagctagggcttcccgccatcggcaagacggagaagaccggcaagcgctccaccagcgccgccgtcctggaggccctccgcgaggcccaccccatcgtggagaagatcctgcagtaccgggagctcaccaagctgaagagcacctacattgaccccttgccggacctcatccaccccaggacgggccgcctccacacccgcttcaaccagacggccacggccacgggcaggctaagtagctccgatcccaacctccagaacatccccgtccgcaccccgcttgggcagaggatccgccgggccttcatcgccgaggaggggtggctattggtggccctggactatagccagatagagctcagggtgctggcccacctctccggcgacgagaacctgatccgggtcttccaggaggggcgggacatccacacggagaccgccagctggatgttcggcgtcccccgggaggccgtggaccccctgatgcgccgggcggccaagaccatcaacttcggggtcctctacggcatgtcggcccaccgcctctcccaggagctagccatcccttacgaggaggcccaggccttcattgagcgctactttcagagcttccccaaggtgcgggcctggattgagaagaccctggaggagggcaggaggcgggggtacgtggagaccctcttcggccgccgccgctacgtgccagacctagaggcccgggtgaagagcgtgcgggaggcggccgagcgcatggccttcaacatgcccgtccagggcaccgccgccgacctcatgaagctggctatggtgaagctcttccccaggctggaggaaatgggggccaggatgctccttcaggtccacgacgagctggtcctcgaggccccaaaagagagggcggaggccgtggcccggctggccaaggaggtcatggagggggtgtatcccctggccgtgcccctggaggtggaggtggggataggggaggactggctctccgccaaggagtgatagatctga

SEQ ID NO: 5 - DNA, 2829 bp, Artificial Sequence
  source: /note="Description of Artificial Sequence: Synthetic polynucleotide"
acacaggaaacagcgatgatcgacctgcagcggccgcaggccgccaccatggactctagacaccatcaccatcaccacccatgggattacaaggacgacgatgacaagccgcggtggaattcgagcgcaaccgtaaagttcaagtacaaaggcgaagaaaaagaggtagacatctccaagatcaagaaagtatggcgtgtgggcaagatgatctccttcacctacgacgagggcggtggcaagaccggccgcggtgcggtaagcgaaaaggacgcgccgaaggagctgctgcagatgctggagaagcagaaaaagattaagaattcgggtaacctgcccctctttgagcccaagggccgggtcctcctggtggacggccaccacctggcctaccgcaccttccacgccctgaagggcctcaccaccagccggggggagccggtgcaggcggtctacggcttcgccaagagcctcctcaaggccctcaaggaggacggggacgcggtgatcgtggtctttgacgccaaggccccctccttccgccacgaggcctacggggggtacaaggcgggccgggcccccacaccggaggactttccccggcaactcgccctcatcaaggagctggtggacctcctggggctggcgcgcctcgaggtcccgggctacgaggcggacgacgtcctggccagcctggccaagaaggcggaaaaggagggctacgaggtccgcatcctcaccgccgacaaagacctttaccagctcctttccgaccgcatccacgtcctccaccccgaggggtacctcatcaccccggcctggctttgggaaaagtacggcctgaggcccgaccagtgggccgactaccgggccctgaccggggacgagtccgacaaccttcccggggtcaagggcatcggggagaagacggcgaggaagcttctggaggagtgggggagcctggaagccctcctcaagaacctggaccggctgaagcccgccatccgggagaagatcctggcccacatggacgatctgaagctctcctgggacctggccaaggtgcgcaccgacctgcccctggaggtggacttcgccaaaaggcgggagcccgaccgggagaggcttagggcctttctggagaggcttgagtttggcagcctcctccacgagttcggccttctggaaagccccaaggccctggaggaggccccctggcccccgccggaaggggccttcgtgggctttgtgctttcccgcaaggagcccatgtgggccgatcttctggccctggccgccgccagggggggccgggtccaccgggcccccgagccttataaagccctcagggacctgaaggaggcgcgggggcttctcgccaaagacctgagcgttctggccctgagggaaggccttggcctcccgcccggcgacgaccccatgctcctcgcctacctcctggacccttccaacaccacccccgagggggtggcccggcgctacggcggggagtggacggaggaggcgggggagcgggccgccctttccgagaggctcttcgccaacctgtgggggaggcttgagggggaggagaggctcctttggctttaccgggaggtggagaggcccctttccgctgtcctggcccacatggaggccacgggggtgcgcctggacgtggcctatctcagggccttgtccctggaggtggccgaggagatcgcccgcctcgaggccgaggtcttccgcctggccggccaccccttcaacctcaactcccgggaccagctggaaagggtcctctttgacgagctagggcttcccgccatcggcaagacggagaagaccggcaagcgctccaccagcgccgccgtcctggaggccctccgcgaggcccaccccatcgtggagaagatcctgcagtaccgggagctcaccaagctgaagagcacctacattgaccccttgccggacctcatccaccccaggacgggccgcctccacacccgcttcaaccagacggccacggccacgggcaggctaagtagctccgatcccaacctccagaacatccccgtccgcaccccgcttgggcagaggatccgccgggccttcatcgccgaggaggggtggctattggtggccctggactatagccagatagagctcagggtgctggcccacctctccggcgacgagaacctgatccgggtcttccaggaggggcgggacatccacacggagaccgccagctggatgttcggcgtcccccgggaggccgtggaccccctgatgcgccgggcggccaagaccatcaacttcggggtcctctacggcatgtcggcccaccgcctctcccaggagctagccatcccttacgaggaggcccaggccttcattgagcgctactttcagagcttccccaaggtgcgggcctggattgagaagaccctggaggagggcaggaggcgggggtacgtggagaccctcttcggccgccgccgctacgtgccagacctagaggcccgggtgaagagcgtgcgggaggcggccgagcgcatggccttcaacatgcccgtccagggcaccgccgccgacctcatgaagctggctatggtgaagctcttccccaggctggaggaaatgggggccaggatgctccttcaggtccacgacgagctggtcctcgaggccccaaaagagagggcggaggccgtggcccggctggccaaggaggtcatggagggggtgtatcccctggccgtgcccctggaggtggaggtggggataggggaggactggctctccgccaaggagtgatagatctga

SEQ ID NO: 6 - protein, 934 aa, Artificial Sequence
  source: /note="Description of Artificial Sequence: Synthetic polypeptide"
MIDLQRPQAATMDSRHHHHHHPWDYKDDDDKPRWNSSATVKFKYKGEEKEVDISKIKKVWRVGKMISFTYDEGGGKTGRGAVSEKDAPKELLQMLEKQKKIKNSGNLPLFEPKGRVLLVDGHHLAYRTFHALKGLTTSRGEPVQAVYGFAKSLLKALKEDGDAVIVVFDAKAPSFRHEAYGGYKAGRAPTPEDFPRQLALIKELVDLLGLARLEVPGYEADDVLASLAKKAEKEGYEVRILTADKDLYQLLSDRIHVLHPEGYLITPAWLWEKYGLRPDQWADYRALTGDESDNLPGVKGIGEKTARKLLEEWGSLEALLKNLDRLKPAIREKILAHMDDLKLSWDLAKVRTDLPLEVDFAKRREPDRERLRAFLERLEFGSLLHEFGLLESPKALEEAPWPPPEGAFVGFVLSRKEPMWADLLALAAARGGRVHRAPEPYKALRDLKEARGLLAKDLSVLALREGLGLPPGDDPMLLAYLLDPSNTTPEGVARRYGGEWTEEAGERAALSERLFANLWGRLEGEERLLWLYREVERPLSAVLAHMEATGVRLDVAYLRALSLEVAEEIARLEAEVFRLAGHPFNLNSRDQLERVLFDELGLPAIGKTEKTGKRSTSAAVLEALREAHPIVEKILQYRELTKLKSTYIDPLPDLIHPRTGRLHTRFNQTATATGRLSSSDPNLQNIPVRTPLGQRIRRAFIAEEGWLLVALDYSQIELRVLAHLSGDENLIRVFQEGRDIHTETASWMFGVPREAVDPLMRRAAKTINFGVLYGMSAHRLSQELAIPYEEAQAFIERYFQSFPKVRAWIEKTLEEGRRRGYVETLFGRRRYVPDLEARVKSVREAAERMAFNMPVQGTAADLMKLAMVKLFPRLEEMGARMLLQVHDELVLEAPKERAEAVARLAKEVMEGVYPLAVPLEVEVGIGEDWLSAKE

SEQ ID NO: 7 - DNA, 325 bp, Artificial Sequence
  source: /note="Description of Artificial Sequence: Synthetic polynucleotide"
atgatcgacctgcagcggccgcaggccgccaccatggactctagacaccatcaccatcaccacccatgggattacaaggacgacgatgacaagccgcggtggaattcgagcgcaaccgtaaagttcaagtacaaaggcgaagaaaaagaggtagacatctccaagatcaagaaagtatggcgtgtgggcaagatgatctccttcacctacgacgagggcggtggcaagaccggccgcggtgcggtaagcgaaaaggacgcgccgaaggagctgctgcagatgctggagaagcagaaaaagattaagaattcgggtaacctgcccc

SEQ ID NO: 8 - protein, 106 aa, Artificial Sequence
  source: /note="Description of Artificial Sequence: Synthetic polypeptide"
MIDLQRPQAATMDSRHHHHHHPWDYKDDDDKPRWNSSATVKFKYKGEEKEVDISKIKKVWRVGKMISFTYDEGGGKTGRGAVSEKDAPKELLQMLEKQKKIKNSGN

SEQ ID NO: 9 - DNA, 204 bp, Artificial Sequence
  source: /note="Description of Artificial Sequence: Synthetic polynucleotide"
agcgcaaccgtaaagttcaagtacaaaggcgaagaaaaagaggtagacatctccaagatcaagaaagtatggcgtgtgggcaagatgatctccttcacctacgacgagggcggtggcaagaccggccgcggtgcggtaagcgaaaaggacgcgccgaaggagctgctgcagatgctggagaagcagaaaaagattaagaattcg

SEQ ID NO: 10 - protein, 68 aa, Artificial Sequence
  source: /note="Description of Artificial Sequence: Synthetic polypeptide"
SATVKFKYKGEEKEVDISKIKKVWRVGKMISFTYDEGGGKTGRGAVSEKDAPKELLQMLEKQKKIKNS

SEQ ID NO: 11 - protein, 876 aa, Artificial Sequence
  source: /note="Description of Artificial Sequence: Synthetic polypeptide"
MIDLQRPQAATMDSRHHHHHHPWDYKDDDDKPRWNSILDTDYITEDGKPVIRIFKKENGEFKIDYDRNFEPYIYALLKDDSAIEDVKKITAERHGTTVRVVRAEKVKKKFLGRPIEVWKLYFTHPQDVPAIRDKIKEHPAVVDIYEYDIPFAKRYLIDKGLIPMEGDEELKMLAFDIETLYHEGEEFAEGPILMISYADEEGARVITWKNIDLPYVDVVSTEKEMIKRFLKVVKEKDPDVLITYNGDNFDFAYLKKRSEKLGVKFILGREGSEPKIQRMGDRFAVEVKGRIHFDLYPVIRRTINLPTYTLEAVYEAIFGQPKEKVYAEEIAQAWETGEGLERVARYSMEDAKVTYELGKEFFPMEAQLSRLVGQSLWDVSRSSTGNLVEWFLLRKAYERNELAPNKPDERELARRRESYAGGYVKEPERGLWENIVYLDFRSLYPSIIITHNVSPDTLNREGCEEYDVAPQVGHKFCKDFPGFIPSLLGDLLEERQKVKKKMKATIDPIEKKLLDYRQRAIKILANSFYGYYGYAKARWYCKECAESVTAWGRQYIETTIREIEEKFGFKVLYADTDGFFATIPGADAETVKKKAKEFLDYINAKLPGLLELEYEGFYKRGFFVTKKKYAVIDEEDKITTRGLEIVRRDWSEIAKETQARVLEAILKHGDVEEAVRIVKEVTEKLSKYEVPPEKLVIYEQITRDLKDYKATGPHVAVAKRLAARGIKIRPGTVISYIVLKGSGRIGDRAIPFDEFDPAKHKYNAEYYIENQVLPAVERILRAFGYRKEDLRYQKTRQVGLGAWLKPKTSWICATVKFKYKGEEKEVDISKIKKVWRVGKMISFTYDEGGGKTGRGAVSEKDAPKELLQMLEKQKKI

SEQ ID NO: 12 - DNA, 2634 bp, Artificial Sequence
  source: /note="Description of Artificial Sequence: Synthetic polynucleotide"
atgatcgacctgcagcggccgcaggccgccaccatggactctagacaccatcaccatcaccacccatgggattacaaggacgacgatgacaagccgcggtggaattccatcctcgatacagactacataactgaggatggaaagcccgtcatcaggatcttcaagaaggagaacggcgagttcaaaatagactacgacagaaactttgagccatacatctacgcgctcttgaaggacgactctgcgattgaggacgtcaagaagataactgccgagaggcacggcactaccgttagggttgtcagggccgagaaagtgaagaagaagttcctaggcaggccgatagaggtctggaagctctacttcactcacccccaggacgttcccgcaatcagggacaagataaaggagcatcctgccgttgtggacatctacgagtacgacatccccttcgcgaagcgctacctcatagacaaaggcttaatcccgatggagggcgacgaggaacttaagatgctcgccttcgacatcgagacgctctatcacgagggcgaggagttcgccgaagggcctatcctgatgataagctacgccgacgaggaaggggcgcgcgttattacctggaagaatatcgaccttccctatgtcgacgtcgtttccaccgagaaggagatgataaagcgcttcctcaaggtcgtcaaggaaaaggatcccgacgtcctcataacctacaacggcgacaacttcgacttcgcctacctcaagaagcgctccgagaagctcggagtcaagttcatcctcggaagggaagggagcgagccgaaaatccagcgcatgggcgatcgctttgcggtggaggtcaagggaaggattcacttcgacctctaccccgtcattaggagaacgattaacctccccacttacacccttgaggcagtatatgaagccatctttggacagccgaaggagaaggtctacgctgaggagatagcgcaggcctgggaaacgggcgagggattagaaagggtggcccgctactcgatggaggacgcaaaggtaacctatgaactcggaaaagagttcttccctatggaagcccagctctcgcgcctcgtaggccagagcctctgggatgtatctcgctcgagtaccggaaacctcgtcgagtggtttttgctgaggaaggcctacgagaggaatgaacttgcaccaaacaagccggacgagagggagctggcaagaagaagggagagctacgcgggtggatacgtcaaggagcccgaaaggggactgtgggagaacatcgtgtatctggacttccgctccctgtatccttcgataataatcacccataacgtctcccctgatacactcaacagggagggttgtgaggagtacgacgtggctcctcaggtaggccataagttctgcaaggacttccccggcttcatcccaagcctcctcggggacctcttggaggagagacagaaggtaaagaagaagatgaaggccactatagacccaatcgagaagaaactcctcgattacaggcagcgagcaatcaaaatccttgctaatagcttctacggttactacggctatgcaaaggcccgctggtactgcaaggagtgcgccgagagcgttaccgcttggggcaggcagtacatcgagaccacgataagggaaatagaggagaaatttggctttaaagtcctctacgcggacacagatggatttttcgcaacaatacctggagcggacgccgaaaccgtcaaaaagaaggcaaaggagttcctggactacatcaacgccaaactgcccggcctgctcgaactcgaatacgagggcttctacaagcgcggcttcttcgtgacgaagaagaagtacgcggttatagacgaggaggacaagataacgacgcgcgggcttgaaatagttaggcgtgactggagcgagatagcgaaggagacgcaggcgagggttcttgaggcgatactaaagcacggtgacgttgaagaagcggtaaggattgtcaaagaggttacggagaagctgagcaagtacgaggttccaccggagaagctggtcatctacgagcagataacccgcgacctgaaggactacaaggccaccgggccgcatgtggctgttgcaaaacgcctcgccgcaagggggataaaaatccggcccggaacggtcataagctacatcgtgctcaaaggctcgggaaggattggggacagggctataccctttgacgaatttgacccggcaaagcacaagtacaatgcagaatactacatcgagaaccaggttcttccagctgtggagaggattctgagggcctttggttaccgtaaagaagatttaaggtatcagaaaacgcggcaggttggcttgggggcgtggctaaaacctaagacaagctggatctgcgcaaccgtaaagttcaagtacaaaggcgaagaaaaagaggtagacatctccaagatcaagaaagtatggcgtgtgggcaagatgatctccttcacctacgacgagggcggtggcaagaccggccgcggtgcggtaagcgaaaaggacgcgccgaaggagctgctgcagatgctggagaagcagaaaaagatttagtgg

SEQ ID NO: 13 - protein, 31 aa, Artificial Sequence
  source: /note="Description of Artificial Sequence: Synthetic polypeptide"
MVDDLQRPHHHHHHPWDYKDDDDKPRWNSGW

SEQ ID NO: 14 - protein, 36 aa, Artificial Sequence
  source: /note="Description of Artificial Sequence: Synthetic polypeptide"
MIDLQRPQAATMDSRHHHHHHPWDYKDDDDKPRWNS

SEQ ID NO: 15 - DNA, 108 bp, Artificial Sequence
  source: /note="Description of Artificial Sequence: Synthetic polynucleotide"
atgatcgacctgcagcggccgcaggccgccaccatggactctagacaccatcaccatcaccacccatgggattacaaggacgacgatgacaagccgcggtggaattcc

SEQ ID NO: 16 - protein, 40 aa, Artificial Sequence
  source: /note="Description of Artificial Sequence: Synthetic polypeptide"
MIDLQRPSAATMVDDLQRPHHHHHHPWDYKDDDDKPRWNS

SEQ ID NO: 17 - DNA, 120 bp, Artificial Sequence
  source: /note="Description of Artificial Sequence: Synthetic polynucleotide"
atgatcgacctgcagcggccatccgccgccaccatggtcgacgacctgcagcggccgcaccatcaccatcaccatccatgggattacaaggacgacgatgacaagccgcggtggaattcg

SEQ ID NO: 18 - protein, 29 aa, Artificial Sequence
  source: /note="Description of Artificial Sequence: Synthetic peptide"
MVDDLQRPHHHHHHPWDYKDDDDKPRWNS

SEQ ID NO: 19 - DNA, 87 bp, Artificial Sequence
  source: /note="Description of Artificial Sequence: Synthetic oligonucleotide"
atggtcgacgacctgcagcggccgcaccatcaccatcaccatccatgggattacaaggacgacgatgacaagccgcggtggaattcg

SEQ ID NO: 20 - protein, 207 aa, Artificial Sequence
  source: /note="Description of Artificial Sequence: Synthetic polypeptide"
MIDLQRPSAATMVDDLQRPHHHHHHPWDYKDDDDKPRWNSGAPPRLICDSRVLERYLLEAKEAENITTGCAEHCSLNENITVPDTKVNFYAWKRMEVGQQAVEVWQGLALLSEAVLRGQALLVNSSQPWEPLQLHVDKAVSGLRSLTTLLRALGAQKEAISPPDAASAAPLRTITADTFRKLFRVYSNFLRGKLKLYTGEACRTGDR

SEQ ID NO: 21 - DNA, 621 bp, Artificial Sequence
  source: /note="Description of Artificial Sequence: Synthetic polynucleotide"
atgatcgacctgcagcggccatccgccgccaccatggtcgacgacctgcagcggccgcaccatcaccatcaccatccatgggattacaaggacgacgatgacaagccgcggtggaattcgggggccccaccacgcctcatctgtgacagccgagtcctggagaggtacctcttggaggccaaggaggccgagaatatcacgacgggctgtgctgaacactgcagcttgaatgagaatatcactgtcccagacaccaaagttaatttctatgcctggaagaggatggaggtcgggcagcaggccgtagaagtctggcagggcctggccctgctgtcggaagctgtcctgcggggccaggccctgttggtcaactcttcccagccgtgggagcccctgcagctgcatgtggataaagccgtcagtggccttcgcagcctcaccactctgcttcgggctctgggagcccagaaggaagccatctcccctccagatgcggcctcagctgctccactccgaacaatcactgctgacactttccgcaaactcttccgagtctactccaatttcctccggggaaagctgaagctgtacacaggggaggcctgcaggacaggggacaga

SEQ ID NO: 22 - protein, 241 aa, Artificial Sequence
  source: /note="Description of Artificial Sequence: Synthetic polypeptide"
MIDLQRPSAATMVDDLQRPHHHHHHPWDYKDDDDKPRWNSKVLAAGVVPLLLVLHWKHGAGSPLPITPVNATCAIRHPCHNNLMNQIRSQLAQLNGSANALFILYYTAQGEPFPNNLDKLCGPNVTDFPPFHANGTEKAKLVELYRIVVYLGTSLGNITRDQKILNPSALSLHSKLNATADILRGLLSNVLCRLCSKYHVGHVDVTYGPDTSGKDVFQKKKLGCQLLGKYKQIIAVLAQAF

SEQ ID NO: 23 - DNA, 723 bp, Artificial Sequence
  source: /note="Description of Artificial Sequence: Synthetic polynucleotide"
atgatcgacctgcagcggccatccgccgccaccatggtcgacgacctgcagcggccgcaccatcaccatcaccatccatgggattacaaggacgacgatgacaagccgcggtggaattcgaaagtgctggcggcgggcgtggtgccgctgctgctggtgctgcattggaaacatggcgcgggcagcccgctgccgattaccccggtgaacgcgacctgcgcgattcgccatccgtgccataacaacctgatgaaccagattcgcagccagctggcgcagctgaacggcagcgcgaacgcgctgtttattctgtattataccgcgcagggcgaaccgtttccgaacaacctggataaactgtgcggcccgaacgtgaccgattttccgccgtttcatgcgaacggcaccgaaaaagcgaaactggtggaactgtatcgcattgtggtgtatctgggcaccagcctgggcaacattacccgcgatcagaaaattctgaacccgagcgcgctgagcctgcatagcaaactgaacgcgaccgcggatattctgcgcggcctgctgagcaacgtgctgtgccgcctgtgcagcaaatatcatgtgggccatgtggatgtgacctatggcccggataccagcggcaaagatgtgtttcagaaaaaaaaactgggctgccagctgctgggcaaatataaacagattattgcggtgctggcgcaggcgttt

SEQ ID NO: 24 - protein, 6 aa, Artificial Sequence
  source: /note="Description of Artificial Sequence: Synthetic His tag"
  MISC_FEATURE (1)..(6): /note="This sequence may encompass 1-6 His residues"
HHHHHH

SEQ ID NO: 25 - protein, 5 aa, Artificial Sequence
  source: /note="Description of Artificial Sequence: Synthetic peptide"
DDDDK

SEQ ID NO: 26 - DNA, 15 bp, Unknown
  source: /note="Description of Unknown: Eukaryotic Kozak sequence"
gccgccaccatggtc

SEQ ID NO: 27 - protein, 20 aa, Artificial Sequence
  source: /note="Description of Artificial Sequence: Synthetic His tag"
  MISC_FEATURE (1)..(20): /note="This sequence may encompass 1-15 or 20 His residues"
  MISC_FEATURE (1)..(20): /note="See specification as filed for detailed description of substitutions and preferred embodiments"
HHHHHHHHHHHHHHHHHHHH

SEQ ID NO: 28 - DNA, 12 bp, Artificial Sequence
  source: /note="Description of Artificial Sequence: Synthetic oligonucleotide"
  MISC_FEATURE (1)..(12): /note="This sequence may encompass 6-12 dT nucleotides"
tttttttttttt

SEQ ID NO: 29 - DNA, 10 bp, Artificial Sequence
  source: /note="Description of Artificial Sequence: Synthetic oligonucleotide"
tttttttttt

SEQ ID NO: 30 - RNA, 13 nt, Artificial Sequence
  source: /note="Description of Artificial Sequence: Synthetic oligonucleotide"
gccgccrccaugg

SEQ ID NO: 31 - protein, 5 aa, Unknown
  source: /note="Description of Unknown: Eukaryotic translation signal sequence"
MVDDL